European Patent Application EP 4 793 362 A1, published August 19, 2026. Title: Method for ligation, method for suppressing adapter dimer formation, method for preparing NGS library, NGS library preparation kit, and 3' adapter. Applicant: ARKRAY, Inc. The sequence listing filed with the application follows.

SEQUENCE LISTING (11 sequences)

SEQ ID NO: 1 - RNA, 30 nt, synthetic construct
  source 1..30: mol_type = other RNA
gttcagagttctacagtccgacgatcggag

SEQ ID NO: 2 - RNA, 30 nt, synthetic construct
  source 1..30: mol_type = other RNA
gttcagagttctacagtccgacgatccacg

SEQ ID NO: 3 - RNA, 30 nt, synthetic construct
  source 1..30: mol_type = other RNA
gttcagagttctacagtccgacgatcttgt

SEQ ID NO: 4 - RNA, 26 nt, synthetic construct
  source 1..26: mol_type = other RNA
gttcagagttctacagtccgacgatc

SEQ ID NO: 5 - RNA, 30 nt, synthetic construct
  source 1..30: mol_type = other RNA
gttcagagttctacagtccgacgatctcat

SEQ ID NO: 6 - RNA, 30 nt, synthetic construct
  source 1..30: mol_type = other RNA
gttcagagttctacagtccgacgatctgca

SEQ ID NO: 7 - DNA, 19 bp, synthetic construct
  source 1..19: mol_type = other DNA
  modified_base 19: mod_base = OTHER; note = modified by dideoxycytidine
  modified_base 1: mod_base = OTHER; note = modified by adenylic acid
nnnngtaggcaccatcaat

SEQ ID NO: 8 - DNA, 61 bp, synthetic construct
  source 1..61: mol_type = other DNA
gtgactggagttcagacgtgtgctcttccgatctnnnnnnnnnnnnattgatggtgcctac

SEQ ID NO: 9 - DNA, 55 bp, synthetic construct
  source 1..55: mol_type = other DNA
caagcagaagacggcatacgagatcgtgatgctccaccgataaatattagcccgt

SEQ ID NO: 10 - DNA, 50 bp, synthetic construct
  source 1..50: mol_type = other DNA
aatgatacggcgaccaccgagatctacacgttcagagttctacagtccga

SEQ ID NO: 11 - DNA, 19 bp, synthetic construct
  source 1..19: mol_type = other DNA
  modified_base 19: mod_base = OTHER; note = modified by dideoxycytidine
  modified_base 1: mod_base = OTHER; note = modified by adenylic acid
aactgtaggcaccatcaat